European Patent Application EP 4 541 366 A1, published April 23, 2025. Title: FOXM1 억제제 및 면역관문 억제제를 포함하는 암의 예방 또는 치료용 약학적 조성물. Applicant: 국립암센터. The sequence listing filed with the application follows.

SEQUENCE LISTING (9 sequences)

SEQ ID NO: 1 - DNA, 24 bp, synthetic construct
  source 1..24: mol_type = other DNA
catgtttgagaccttcaacacccc

SEQ ID NO: 2 - DNA, 23 bp, synthetic construct
  source 1..23: mol_type = other DNA
gccatctcctgctcgaagtctag

SEQ ID NO: 3 - DNA, 20 bp, synthetic construct
  source 1..20: mol_type = other DNA
atctcagcaccactcccttg

SEQ ID NO: 4 - DNA, 20 bp, synthetic construct
  source 1..20: mol_type = other DNA
cttgctgaggctgtcattca

SEQ ID NO: 5 - DNA, 20 bp, synthetic construct
  source 1..20: mol_type = other DNA
tatggtggtgccgactacaa

SEQ ID NO: 6 - DNA, 20 bp, synthetic construct
  source 1..20: mol_type = other DNA
tgcttgtccagatgacttcg

SEQ ID NO: 7 - DNA, 20 bp, synthetic construct
  source 1..20: mol_type = other DNA
caaggtgcgttcagatgttg

SEQ ID NO: 8 - DNA, 20 bp, synthetic construct
  source 1..20: mol_type = other DNA
tcctgaccttcggtgaaatc

SEQ ID NO: 9 - DNA, 42 bp, synthetic construct
  source 1..42: mol_type = other DNA
tcacttcacaccgcatctctacgtccggttgcgctttccttt